European Patent Specification EP 3 885 447 B1, published January 10, 2024. Title: DETECTING HEMATOLOGICAL DISORDERS USING CELL-FREE DNA IN BLOOD. Applicant: The Chinese University Of Hong Kong. The sequence listing filed with the application follows.

SEQUENCE LISTING (24 sequences)

SEQ ID NO: 1 - DNA, 30 bp, Artificial Sequence
  FECH gene primer
tttagtttatagttgaagagaatttgatgg

SEQ ID NO: 2 - DNA, 25 bp, Artificial Sequence
  FECH gene primer
aaacccaaccatacaacctcttaat

SEQ ID NO: 3 - DNA, 26 bp, Artificial Sequence
  Forward primer-1
ttgaagagaatttgatggtatgggta

SEQ ID NO: 4 - DNA, 25 bp, Artificial Sequence
  Forward primer-2
tgaagagaatttgatggtacgggta

SEQ ID NO: 5 - DNA, 27 bp, Artificial Sequence
  Reverse
ctcaaatctctctaatttccaaacaca

SEQ ID NO: 6 - DNA, 17 bp, Artificial Sequence
  Fluorescence probe
  misc_feature (1)..(1): 5' FAM fluorescent reporter
  misc_feature (17)..(17): 3' MGB quencher
ttgtgtggtgtagagag

SEQ ID NO: 7 - DNA, 26 bp, Artificial Sequence
  Forward
ttgaagagaatttgatggtatgggta

SEQ ID NO: 8 - DNA, 25 bp, Artificial Sequence
  Forward
tgaagagaatttgatggtacgggta

SEQ ID NO: 9 - DNA, 25 bp, Artificial Sequence
  Reverse
caaatctctctaatttccgaacacg

SEQ ID NO: 10 - DNA, 14 bp, Artificial Sequence
  Fluorescence probe
  misc_feature (1)..(1): 5' VIC fluorescent reporter
  misc_feature (14)..(14): 3' MGB quencher
tgcgtggcgtagag

SEQ ID NO: 11 - DNA, 26 bp, Artificial Sequence
  Forward primer
  misc_feature (21)..(21): n is a, c, g, or t
ttgaagagaatttgatggtangggta

SEQ ID NO: 12 - DNA, 25 bp, Artificial Sequence
  Reverse primer
caaatctctctaatttccgaacacg

SEQ ID NO: 13 - DNA, 14 bp, Artificial Sequence
  Fluorescence probe
  misc_feature (1)..(1): 5' VIC fluorescent reporter
  misc_feature (14)..(14): 3' MGB quencher
tgcgtggcgtagag

SEQ ID NO: 14 - DNA, 26 bp, Artificial Sequence
  Forward primer
  misc_feature (21)..(21): n is a, c, g, or t
ttgaagagaatttgatggtangggta

SEQ ID NO: 15 - DNA, 27 bp, Artificial Sequence
  Reverse primer
ctcaaatctctctaatttccaaacaca

SEQ ID NO: 16 - DNA, 17 bp, Artificial Sequence
  Fluorescence probe
  misc_feature (1)..(1): 5' FAM fluorescent reporter
  misc_feature (17)..(17): 3' MGB quencher
ttgtgtggtgtagagag

SEQ ID NO: 17 - DNA, 27 bp, Artificial Sequence
  Forward primer
  misc_feature (8)..(8): n is a, c, g, or t
gagtaagnggagttgttggtattatgg

SEQ ID NO: 18 - DNA, 26 bp, Artificial Sequence
  Reverse primer
accctcaacccaactcctaaaataac

SEQ ID NO: 19 - DNA, 17 bp, Artificial Sequence
  Fluorescence probe for methylated sequences
  misc_feature (1)..(1): 5' VIC fluorescent reporter
  misc_feature (17)..(17): 3' MGB quencher
tcgggttaggcgtgcgt

SEQ ID NO: 20 - DNA, 19 bp, Artificial Sequence
  Fluorescence probe for unmethylated sequences
  misc_feature (1)..(1): 5' FAM fluorescent reporter
  misc_feature (19)..(19): 3' MGB quencher
ttgggttaggtgtgtgttt

SEQ ID NO: 21 - DNA, 28 bp, Artificial Sequence
  Forward primer
  misc_feature (22)..(22): n is a, c, g, or t
atgtagagttggtaaagataanggaagg

SEQ ID NO: 22 - DNA, 27 bp, Artificial Sequence
  Reverse primer
cattactaccctaaacaaaaccaaacc

SEQ ID NO: 23 - DNA, 20 bp, Artificial Sequence
  Fluorescence probe for methylated sequences
  misc_feature (1)..(1): 5' VIC fluorescent reporter
  misc_feature (20)..(20): 3' MGB quencher
aaggttcgtagtacgtcgta

SEQ ID NO: 24 - DNA, 21 bp, Artificial Sequence
  Fluorescence probe for unmethylated sequences
  misc_feature (1)..(1): 5' FAM fluorescent reporter
  misc_feature (21)..(21): 3' MGB quencher
aaggtttgtagtatgttgtag